European Patent Specification EP 3 637 422 B1, published December 20, 2023. Title: COMPUTER FILES AND METHODS SUPPORTING FORENSIC ANALYSIS OF NUCLEOTIDE SEQUENCE DATA. Applicant: BATTELLE MEMORIAL INSTITUTE. The sequence listing filed with the application follows.

SEQUENCE LISTING (75 sequences)

SEQ ID NO: 1 - DNA, 35 bp, Homo sapiens
aatgaatgaatgaatgaatgatgaatgaatgaatg

SEQ ID NO: 2 - DNA, 36 bp, Homo sapiens
agatagatagatagatagatagatagatagatagat

SEQ ID NO: 3 - DNA, 40 bp, Homo sapiens
agatagatagatagatagatagatagatagatagatagat

SEQ ID NO: 4 - DNA, 83 bp, Unknown
  Illustrative oligonucleotide
gcagacccataatgtcaatagatgtggtagaagtcgtcatttggcgagaaagctcagtcccaggaggaagcggagcagtccaa

SEQ ID NO: 5 - DNA, 83 bp, Unknown
  Illustrative oligonucleotide
ttccaatcatagccacagtttacaacatttgtatctttatctgtatccttatttatacatctatctatctatctatctatcta

SEQ ID NO: 6 - DNA, 83 bp, Unknown
  Illustrative oligonucleotide
cttcctactggcccataatccagctgtgggagggagccagtggatttggaaaccgacatggcttggccttgcctgcctgcctc

SEQ ID NO: 7 - DNA, 157 bp, Unknown
  Illustrative polynucleotide
ccagggcagtgttccaacctgagtctgccaaggcctagcaggttgctaaccaccctgtgtctcagttttcctacctgtaaaatgaagatattaccagtaactgccttcatagatagaagatagatagattagatggatagatagatagatagataga

SEQ ID NO: 8 - DNA, 157 bp, Unknown
  Illustrative polynucleotide
ccagggcagtgttccaacctgagtctgccaaggactagcaggttgctaaccaccctgtgtctcagttttcctacctgtaaaatgaagatattaacagtaactgccttcatagatagaagatagatagattagatagttagatagatagatagataga

SEQ ID NO: 9 - DNA, 157 bp, Unknown
  Illustrative polynucleotide
ccagggcagtgttccaacctgagtctgccaaggactagcaggttgctaaccaccctgtgtctcagttttcctacctgtaaaatgaagatattaacagtaactgccttcatagatagaagatagatagattagatagatagatagatagatagataga

SEQ ID NO: 10 - DNA, 40 bp, Unknown; identical to SEQ ID NO: 3
  Illustrative oligonucleotide

SEQ ID NO: 11 - DNA, 52 bp, Unknown
  Illustrative oligonucleotide
agatagatagatagatagatagatagatagatagatagatagatagatagat

SEQ ID NO: 12 - DNA, 48 bp, Unknown
  Illustrative oligonucleotide
agatagatagatagatagatagatagatagatagatagatagatagat

SEQ ID NO: 13 - DNA, 36 bp, Unknown; identical to SEQ ID NO: 2
  Illustrative oligonucleotide

SEQ ID NO: 14 - DNA, 20 bp, Unknown
  Illustrative oligonucleotide
agatagatagatagatagat

SEQ ID NO: 15 - DNA, 107 bp, Unknown
  Illustrative polynucleotide
tctatctatctatctatctgtctgtctgtctgtctgtctgtctatctatctatatctatctatctatcatctatctatccatatctatctatctatctatctatcta

SEQ ID NO: 16 - DNA, 12 bp, Unknown
  Illustrative oligonucleotide
tctatctatcta

SEQ ID NO: 17 - DNA, 16 bp, Unknown
  Illustrative oligonucleotide
tctatctatctatcta

SEQ ID NO: 18 - DNA, 20 bp, Unknown
  Illustrative oligonucleotide
tctatctatctatctatctg

SEQ ID NO: 19 - DNA, 24 bp, Unknown
  Illustrative oligonucleotide
tctatctatctatctatctgtctg

SEQ ID NO: 20 - DNA, 28 bp, Unknown
  Illustrative oligonucleotide
tctatctatctatctatctgtctgtctg

SEQ ID NO: 21 - DNA, 32 bp, Unknown
  Illustrative oligonucleotide
tctatctatctatctatctgtctgtctgtctg

SEQ ID NO: 22 - DNA, 36 bp, Unknown
  Illustrative oligonucleotide
tctatctatctatctatctgtctgtctgtctgtctg

SEQ ID NO: 23 - DNA, 40 bp, Unknown
  Illustrative oligonucleotide
tctatctatctatctatctgtctgtctgtctgtctgtctg

SEQ ID NO: 24 - DNA, 44 bp, Unknown
  Illustrative oligonucleotide
tctatctatctatctatctgtctgtctgtctgtctgtctgtcta

SEQ ID NO: 25 - DNA, 48 bp, Unknown
  Illustrative oligonucleotide
tctatctatctatctatctgtctgtctgtctgtctgtctgtctatcta

SEQ ID NO: 26 - DNA, 52 bp, Unknown
  Illustrativ oligonucleotide
tctatctatctatctatctgtctgtctgtctgtctgtctgtctatctatcta

SEQ ID NO: 27 - DNA, 53 bp, Unknown
  Illustrative oligonucleotide
tctatctatctatctatctgtctgtctgtctgtctgtctgtctatctatctat

SEQ ID NO: 28 - DNA, 54 bp, Unknown
  Illustrative oligonucleotide
tctatctatctatctatctgtctgtctgtctgtctgtctgtctatctatctata

SEQ ID NO: 29 - DNA, 58 bp, Unknown
  Illustrative oligonucleotide
tctatctatctatctatctgtctgtctgtctgtctgtctgtctatctatctatatcta

SEQ ID NO: 30 - DNA, 62 bp, Unknown
  Illustrative oligonucleotide
tctatctatctatctatctgtctgtctgtctgtctgtctgtctatctatctatatctatcta

SEQ ID NO: 31 - DNA, 66 bp, Unknown
  Illustrative oligonucleotide
tctatctatctatctatctgtctgtctgtctgtctgtctgtctatctatctatatctatctatcta

SEQ ID NO: 32 - DNA, 67 bp, Unknown
  Illustrative oligonucleotide
tctatctatctatctatctgtctgtctgtctgtctgtctgtctatctatctatatctatctatctat

SEQ ID NO: 33 - DNA, 68 bp, Unknown
  Illustrative oligonucleotide
tctatctatctatctatctgtctgtctgtctgtctgtctgtctatctatctatatctatctatctatc

SEQ ID NO: 34 - DNA, 69 bp, Unknown
  Illustrative oligonucleotide
tctatctatctatctatctgtctgtctgtctgtctgtctgtctatctatctatatctatctatctatca

SEQ ID NO: 35 - DNA, 73 bp, Unknown
  Illustrative oligonucleotide
tctatctatctatctatctgtctgtctgtctgtctgtctgtctatctatctatatctatctatctatcatcta

SEQ ID NO: 36 - DNA, 77 bp, Unknown
  Illustrative oligonucleotide
tctatctatctatctatctgtctgtctgtctgtctgtctgtctatctatctatatctatctatctatcatctatcta

SEQ ID NO: 37 - DNA, 81 bp, Unknown
  Illustrative oligonucleotide
tctatctatctatctatctgtctgtctgtctgtctgtctgtctatctatctatatctatctatctatcatctatctatcca

SEQ ID NO: 38 - DNA, 82 bp, Unknown
  Illustrative oligonucleotide
tctatctatctatctatctgtctgtctgtctgtctgtctgtctatctatctatatctatctatctatcatctatctatccat

SEQ ID NO: 39 - DNA, 83 bp, Unknown
  Illustrative oligonucleotide
tctatctatctatctatctgtctgtctgtctgtctgtctgtctatctatctatatctatctatctatcatctatctatccata

SEQ ID NO: 40 - DNA, 87 bp, Unknown
  Illustrative oligonucleotide
tctatctatctatctatctgtctgtctgtctgtctgtctgtctatctatctatatctatctatctatcatctatctatccatatcta

SEQ ID NO: 41 - DNA, 91 bp, Unknown
  Illustrative oligonucleotide
tctatctatctatctatctgtctgtctgtctgtctgtctgtctatctatctatatctatctatctatcatctatctatccatatctatcta

SEQ ID NO: 42 - DNA, 95 bp, Unknown
  Illustrative oligonucleotide
tctatctatctatctatctgtctgtctgtctgtctgtctgtctatctatctatatctatctatctatcatctatctatccatatctatctatcta

SEQ ID NO: 43 - DNA, 99 bp, Unknown
  Illustrative oligonucleotide
tctatctatctatctatctgtctgtctgtctgtctgtctgtctatctatctatatctatctatctatcatctatctatccatatctatctatctatcta

SEQ ID NO: 44 - DNA, 103 bp, Unknown
  Illustrative polynucleotide
tctatctatctatctatctgtctgtctgtctgtctgtctgtctatctatctatatctatctatctatcatctatctatccatatctatctatctatctatcta

SEQ ID NO: 45 - DNA, 60 bp, Unknown
  Illustrative oligonucleotide
tttctttctttcttttttctctttctttctttctttctttctttctttctccttccttcc

SEQ ID NO: 46 - DNA, 64 bp, Unknown
  Illustrative oligonucleotide
tttctttctttcttttttctctttctttctttctttctttctttctttctttctccttccttcc

SEQ ID NO: 47 - DNA, 65 bp, Unknown
  Illustrative oligonucleotide
tttctttctttcttttttctctttctttctttctttcttttctttctttctttctccttccttcc

SEQ ID NO: 48 - DNA, 66 bp, Unknown
  source: Illustrative oligonucleotide
tttctttctttcttttttctttctttctttctttctttctttctttctttctttctccttccttcc

SEQ ID NO: 49 - DNA, 68 bp, Unknown
  Illustrative oligonucleotide
tttctttctttcttttttctctttctttctttctttctttctttctttctttctttctccttccttcc

SEQ ID NO: 50 - DNA, 72 bp, Unknown
  Illustrative oligonucleotide
tttctttctttcttttttctctttctttctttctttctttctttctttctttctttctttctccttccttcc

SEQ ID NO: 51 - DNA, 74 bp, Unknown
  Illustrative oligonucleotide
tttctttctttcttttttctttctttctttctttctttctttctttctttctttctttctttctccttccttcc

SEQ ID NO: 52 - DNA, 76 bp, Unknown
  Illustrative oligonucleotide
tttctttctttcttttttctctttctttctttctttctttctttctttctttctttctttctttctccttccttcc

SEQ ID NO: 53 - DNA, 78 bp, Unknown
  Illustrative oligonucleotide
tttctttctttcttttttctttctttctttctttctttctttctttctttctttctttctttctttctccttccttcc

SEQ ID NO: 54 - DNA, 80 bp, Unknown
  Illustrative oligonucleotide
tttctttctttcttttttctctttctttctttctttctttctttctttctttctttctttctttctttctccttccttcc

SEQ ID NO: 55 - DNA, 44 bp, Homo sapiens
agatagatagatagatagatagatagatagatagatagatagat

SEQ ID NO: 56 - DNA, 32 bp, Homo sapiens
agatagatagatagatagatagatagatagat

SEQ ID NO: 57 - DNA, 48 bp, Homo sapiens; identical to SEQ ID NO: 12

SEQ ID NO: 58 - DNA, 36 bp, Homo sapiens
agatagatagatagatagatagataggtagatagat

SEQ ID NO: 59 - DNA, 36 bp, Homo sapiens
agatagatagatagatagatagatagatagataggt

SEQ ID NO: 60 - DNA, 40 bp, Homo sapiens
agatagatagatagatagatagatagataggtagatagat

SEQ ID NO: 61 - DNA, 40 bp, Homo sapiens
agatagatagatagatagatagatagatagataggtagat

SEQ ID NO: 62 - DNA, 40 bp, Homo sapiens
agataggtagatagatagatagatagatagatagatagat

SEQ ID NO: 63 - DNA, 7 bp, Homo sapiens
gatatat

SEQ ID NO: 64 - DNA, 40 bp, Homo sapiens
agatagatcgatagatagctagatagatcgatagatagat

SEQ ID NO: 65 - DNA, 36 bp, Homo sapiens
agatagatagttagatagatagttagatagatagat

SEQ ID NO: 66 - DNA, 36 bp, Homo sapiens
agatagatagatggatagataggtagatggatagat

SEQ ID NO: 67 - DNA, 32 bp, Homo sapiens
agatagatagatagatagatagatggttagat

SEQ ID NO: 68 - DNA, 40 bp, Homo sapiens
agatagatagttagttagatagatagatagttagttagat

SEQ ID NO: 69 - DNA, 36 bp, Homo sapiens
agatagatagatagatagttagttagttagatagat

SEQ ID NO: 70 - DNA, 44 bp, Homo sapiens
agatagatagatagatagttagatagatagatagatagatagat

SEQ ID NO: 71 - DNA, 36 bp, Homo sapiens
agatagatagatagatagacagatagatagttagat

SEQ ID NO: 72 - DNA, 40 bp, Homo sapiens
agatagatagatagttagatagttagatagatagatagat

SEQ ID NO: 73 - DNA, 12 bp, Homo sapiens
attaagtcgtaa

SEQ ID NO: 74 - DNA, 12 bp, Homo sapiens
ctcccagggacg

SEQ ID NO: 75 - DNA, 12 bp, Homo sapiens
ctgtctctctgt